European Patent Specification EP 3 592 851 B1, published November 27, 2024. Title: Method for discovery of alternative antigen specific antibody variants. Applicant: F. Hoffmann-La Roche AG. The sequence listing filed with the application follows.

SEQUENCE LISTING (80 sequences)

SEQ ID NO: 1 - protein, 16 aa, Oryctolagus cuniculus
DHDTGSHPYNYENMDV

SEQ ID NO: 2 - protein, 16 aa, Oryctolagus cuniculus
DHDTGSHPYSYENMDV

SEQ ID NO: 3 - protein, 16 aa, Oryctolagus cuniculus
DHDTGSSPYNYDNMDV

SEQ ID NO: 4 - protein, 16 aa, Oryctolagus cuniculus
DHDTGSSQYNYDNMDV

SEQ ID NO: 5 - protein, 16 aa, Oryctolagus cuniculus
DHDTGSNPYNYDNMDV

SEQ ID NO: 6 - protein, 16 aa, Oryctolagus cuniculus
DHDTGSSPYNYDNMDV

SEQ ID NO: 7 - protein, 16 aa, Oryctolagus cuniculus
DHDTGSHPYKYANMDV

SEQ ID NO: 8 - protein, 16 aa, Oryctolagus cuniculus
EHDTGSHPYCYENMDV

SEQ ID NO: 9 - protein, 16 aa, Oryctolagus cuniculus
DHDTGNHPYNYENMDV

SEQ ID NO: 10 - protein, 16 aa, Oryctolagus cuniculus
DHDTGSHPYSYENMYV

SEQ ID NO: 11 - protein, 16 aa, Oryctolagus cuniculus
DHDTGSHPYSYENMDF

SEQ ID NO: 12 - protein, 16 aa, Oryctolagus cuniculus
DHETGSHPYSYENMDV

SEQ ID NO: 13 - protein, 16 aa, Oryctolagus cuniculus
EHDTGSHPYSYENMDV

SEQ ID NO: 14 - protein, 16 aa, Oryctolagus cuniculus
DHDTGSHPYSYDNMDV

SEQ ID NO: 15 - protein, 16 aa, Oryctolagus cuniculus
DHDTGSHPYSYENIDV

SEQ ID NO: 16 - protein, 16 aa, Oryctolagus cuniculus
DNDTGSHPYSYENMDV

SEQ ID NO: 17 - protein, 16 aa, Oryctolagus cuniculus
DHDNGSHPYSYENMDV

SEQ ID NO: 18 - protein, 16 aa, Oryctolagus cuniculus
DHDTGSHPYSHENMDV

SEQ ID NO: 19 - protein, 16 aa, Oryctolagus cuniculus
DHDTGCHPYSYENMDV

SEQ ID NO: 20 - protein, 16 aa, Oryctolagus cuniculus
DHDTGNHPYSYENMDV

SEQ ID NO: 21 - protein, 16 aa, Oryctolagus cuniculus
DHDTGSHPYSYENMDV

SEQ ID NO: 22 - protein, 16 aa, Oryctolagus cuniculus
DYDTGSHPYNYENMDV

SEQ ID NO: 23 - protein, 16 aa, Oryctolagus cuniculus
DHDTGSHPYNYENLDV

SEQ ID NO: 24 - protein, 16 aa, Oryctolagus cuniculus
DHDTGSHPYNYENRDV

SEQ ID NO: 25 - protein, 16 aa, Oryctolagus cuniculus
DHDTGSHPYNNENMDV

SEQ ID NO: 26 - protein, 16 aa, Oryctolagus cuniculus
DHDTGSHPYNYENMDV

SEQ ID NO: 27 - protein, 16 aa, Oryctolagus cuniculus
DHDTGSSPDNYDNMEV

SEQ ID NO: 28 - protein, 16 aa, Oryctolagus cuniculus
DHDAGSSPYNYDNMDV

SEQ ID NO: 29 - protein, 16 aa, Oryctolagus cuniculus
DSLSYGYAYATNYFNI

SEQ ID NO: 30 - DNA, 37 bp, Artificial Sequence
  rbHC.up
aagcttgccaccatggagactgggctgcgctggcttc

SEQ ID NO: 31 - DNA, 21 bp, Artificial Sequence
  rbHC.do
ccattggtgagggtgcccgag

SEQ ID NO: 32 - DNA, 34 bp, Artificial Sequence
  rbLC.up
aagcttgccaccatggacaygagggcccccactc

SEQ ID NO: 33 - DNA, 26 bp, Artificial Sequence
  rbLC.do
cagagtrctgctgaggttgtaggtac

SEQ ID NO: 34 - DNA, 25 bp, Artificial Sequence
  rbHCfinal_FS.up
atggagactgggctgcgctggcttc

SEQ ID NO: 35 - DNA, 17 bp, Artificial Sequence
  rbHC_shortCH1_fs2.do
gggaagactgatggagc

SEQ ID NO: 36 - protein, 115 aa, Oryctolagus cuniculus
CQSVEESGGRLVTPGTPLTLTCTASGFSLSSYNMNWVRQAPGKGLEWIGYINKGGSAYYASWAKGRFTISRTSTTVDLKMTSPTTEDTATYFCVRSGGGGNLNLWGQGTLVTVSS

SEQ ID NO: 37 - protein, 115 aa, Oryctolagus cuniculus
CQSVEESGGRLVTPGTPLTLTCTASGFSLSSYNMNWVRQAPGKGLEWIGYINKGGSAYYASWAKGRFTISRTSTTVDLKMTSPTPEDTATYFCVRSGGGGNLNLWGQGTLVTVSS

SEQ ID NO: 38 - protein, 115 aa, Oryctolagus cuniculus
CQSVEESGGRLVTPGTPLTLTCTASGFSLSSYNMNWVRQAPGKGLAWIGYINKGGSAYYASWAKGRFTISKTSTTVDLKMTSPTTEDTATYFCVRSGGGGNLNLWGQGTLVTVSS

SEQ ID NO: 39 - protein, 115 aa, Oryctolagus cuniculus
CPPVEESGGRLVTPGTPLTLTCTAPGFSLSSSNMNWVRQAPGKGLEWIGYINKGGSAYYASWAKGRFTISKTSTTVDLKMTSPTTEDTATYFCVRSGGGGNLNLWGQGTLVTVSS

SEQ ID NO: 40 - protein, 115 aa, Oryctolagus cuniculus
CQSVEESGGRLVTPGTPLTLTCTASGFSLSSYNMNWVRQAPGKGLEWIGYINKGGSAYDANWAKGRFTISRTSTTVDLKMTSPTPEDTATYFCVRSGGGGNLNLWGQGTLVTVSS

SEQ ID NO: 41 - protein, 110 aa, Oryctolagus cuniculus
AAVLTQTPSPVSAAVGGTVTISCQSSPNILGNYLSWFQQKPGQPPKLLIYYTSTLASGVPSRFKGSGSGTQFTLTISDVQCDDAATYYCLGVYRSDSDNVFGGGTEVVVK

SEQ ID NO: 42 - protein, 115 aa, Oryctolagus cuniculus
CQLVEESGGRLVTPGTPLTLTCTASGFSLSSYKMNWVRQAPGKGLEWIGYINKGGSAYYASWAKGRFTISRTSTTVDLKMTSPTPEDTATYVCGRSGGGGNLNLWGQGTLVTVSS

SEQ ID NO: 43 - protein, 115 aa, Oryctolagus cuniculus
CQSVEESGGRLVTPGTPLTLTCTASGFSLSSYNMNWVRQAPGKGLEWIGYINKGGSAYYASWAKGRFTISKTSTTVDLKMTSPTTEDTATYFCVRSGGGGNLNLWGQGTLVTVSS

SEQ ID NO: 44 - protein, 116 aa, Oryctolagus cuniculus
CQSVEESGGRLVTPGTPLTLTCTVSGIDLSRSAVGWFRQAPGKGLEYIGFIGSSGTTYCATWAKGRFTISKASTTVALKITSPTTEDTATYFCASRNYDDYTFDPWGPGTLVTVSS

SEQ ID NO: 45 - protein, 116 aa, Oryctolagus cuniculus
CQSVEESGGRLVTPGTPLTLTCTVSGIDLSSYAVGWFRQAPGKGLEYIGFIGSSGTTYYATWAKGRFTISKASTTVSLKMTSPTTEDTATYFCASRNYDDYTFDPWGPGTLVTVSS

SEQ ID NO: 46 - protein, 116 aa, Oryctolagus cuniculus
CQSVEESGGRLVTPGTPLTLTCTVSGIDLSRFAVGWFRQAPGKGLEYIGFIGSSGSTYYASWAKGRFTISKSSTTVDLKIPGPTTEDTATYFCASRNYDDYSFDSWGPGTLVTVAS

SEQ ID NO: 47 - protein, 116 aa, Oryctolagus cuniculus
CQSVEESGGRLVTPGTPLTLTCTVSGIDLSRFAVGWFRQAPGKGLEYIGFIGSSGSTYYASWAKGRFTISKSSTTVDLKMPGPTTEDTATYFCASRNYDDYSFDSWGPGTLVTVSS

SEQ ID NO: 48 - protein, 116 aa, Oryctolagus cuniculus
CQSVEESGGRLVTPGTPLTLTCTVSGIDLSRFAVGWFRQAPGKGLEYIGFIGSSGSTYYASWAKGRFTISKASTTVDLKMPGPTTEDTATYFCASRNYDDYSFDSWGPGTLVTVAS

SEQ ID NO: 49 - protein, 116 aa, Oryctolagus cuniculus
CQSVEESGGRLVTPGTPLTLTCTVSGIDLSRFAVGWFRQAPGKGLEYIGFIGSSGSTYYASWAKGRFTISKSSTTVDLKMPGPTTEDTATYFCASRNYDDYSFDPWGPGTLVTVAS

SEQ ID NO: 50 - protein, 116 aa, Oryctolagus cuniculus
CQSVEESGGRLVTPGTPLTLTCTVSGIDLSRFAVGWFRQAPGKGLEYIGFIGSSGSTYYASWAKGRFTISKSSTTVDLKMPSPTTEDTATYFCASRNYDDYSFDSWGPGTLVTVAS

SEQ ID NO: 51 - protein, 116 aa, Oryctolagus cuniculus
CQSVEESGGRLVTPGTPLTLTCTVSGIDLSRFAVGWFRQAPGKGLEYIGFIGSSGSTYYASWAKGRFTISKSSTTVDLKMTGPTTEDTATYFCASRNYDDYSFDSWGPGTLVTVAS

SEQ ID NO: 52 - protein, 116 aa, Oryctolagus cuniculus
CQSVEESGGRLVTPGTPLTLTCTVSGIDLSSYAVGWLRQAPGKGLEYIGFIGSSGTTYYATWAKGRFTISKASTTVSLKMTSPTTEDTATYFCASRNYDDYTFDPWGPGTLVTVSS

SEQ ID NO: 53 - protein, 116 aa, Oryctolagus cuniculus
CQSVEESGGRLVTPGTPLTLTCTVSGIDLSSYAVGWFRQAPGKGLEYIGFFGSSGTTYYATWAKGRFTISKASTTVSLKMTSPTTEDTATYFCASRNYDDYTFDPWGPGTLVTVSS

SEQ ID NO: 54 - protein, 116 aa, Oryctolagus cuniculus
CQSVEESGGRLVTPGTPLTLTCTVSGIDLSRSAVGWFRQAPGKGLEYIGFIGSSGSTYYASWAKGRFTISKSSTTVDLKMPGPTTEDTATYFCASRNYDDYSFDSWGPGTLVTVAS

SEQ ID NO: 55 - protein, 116 aa, Oryctolagus cuniculus
CQSVEESGGRLVTPGTPLTLTCTVSGIDLSSYAVGWFRQAPGKGLEYIGFIGSSGTTYYATWGKGRFTISNASTTVSLKMTSPTTEDTATYFCASRNYDDYTFDPWGPGTLVTVSS

SEQ ID NO: 56 - protein, 116 aa, Oryctolagus cuniculus
CQSVEESGGRLVTPGTPLTLTCTVSGIDLSRFAVGWFRQAPGKGLEYIGFIGSSGSTYYASWAKGRFTISKSSTTVDLKMTSLTTEDTATYFCASRNYDDYSFDSWGPGTLVTVAS

SEQ ID NO: 57 - protein, 116 aa, Oryctolagus cuniculus
CQSVEESGGRLVTPGTPLTLTCTVSGIDLSSYAVGWFRQAPGKGLEYIGFIGTSGTTYYATWAKGRFTISKASTTVSLKMTSPTTEDTATYFCASRNYDDYTFDPWGPGTLVTVSS

SEQ ID NO: 58 - protein, 116 aa, Oryctolagus cuniculus
CQSVEESGGRLVTPGTPLTLTCTVSGIDLSSYAVGWFRQAPGKGLEYIGFIGSSGTTYYANWAKGRFTISKASTTVSLKMTSPTTEDTATYFCASRNYDDYTFDPWGPGTLVTVSS

SEQ ID NO: 59 - protein, 116 aa, Oryctolagus cuniculus
CQSVEESGGRLVTPGTPLTLTCTVSGIDLSRFAVGWFRQAPGKGLEYIGFIGSSGTTYYASWAKGRFTISKSSTTVDLKMPGPTTEDTATYFCASRNYDDYSFDSWGPGTLVTVAS

SEQ ID NO: 60 - protein, 113 aa, Oryctolagus cuniculus
CQSVEESGGRLVTPGTPLTLTCTVSGFSLSAYVVSWVRQVPGEGLEWIGSLIFDSNRYYASWAKGRFTISKTSTTVDLTITSPTTEDTATYFCARGGYACDLWGQGTLVTVSS

SEQ ID NO: 61 - protein, 113 aa, Oryctolagus cuniculus
CQSVEESGGRLVAPGTPLTLTCTVSGFSLSAYVVSWVRQVPGEGLEWIGSLIFDSNRYYASWAKGRFTISKTSTTVDLTITSPTIEDTATYFCARGGYASDLWGQGTLVTVSS

SEQ ID NO: 62 - protein, 113 aa, Oryctolagus cuniculus
CQSVEESGGRLVTPGTPLTLTCTVSGFSLSAYVVSWVRQVPGEGLEWIGSLIFDSNRYYASWAKGRFTISKTSTTVDLTITSPTIEDTATYFCARGGYASDLWGQGTLVTVSS

SEQ ID NO: 63 - protein, 113 aa, Oryctolagus cuniculus
CQSVEESGGRLVTPGTPLTLTCTVSGFSLSAYVVSWVRQVPGEGLEWIGSLIFDSNRYYASWAKGRFTISKTSTTVDLTITSPTIEDTATYFCARGWTYLDLWGQGTLVTVSS

SEQ ID NO: 64 - protein, 113 aa, Oryctolagus cuniculus
CQSVEESGGRLVTPGTPLTLTCTVSGFSLSAYVVSWVRQVPGEGLEWIGSLIFDSNRYYASWAKGRFTISKTSTTVDPTITSPTIEDTATYFCARGGYASDLWGQGTLVTVSS

SEQ ID NO: 65 - protein, 113 aa, Oryctolagus cuniculus
CQSVEESGGRLVTPGTPLTLTCTVSGFSLSAYVVSWVRQVPGEGLEWIGSLVFDTNTFYASWAKGRFTISKTSPTVDLTITSPTTEDTATYFCTRGGYASDLWGQGTLVTVSS

SEQ ID NO: 66 - protein, 116 aa, Oryctolagus cuniculus; identical to SEQ ID NO: 44

SEQ ID NO: 67 - protein, 120 aa, Oryctolagus cuniculus
CQSLEESGGRLVTPGTPLTLTCTVSGIDLNNDYMTWVRQAPGKGLEWIGIFYVATEITWYASWAKGRFTISKTSTTVDLKITSPTTEDTATYFCGRDGGYTGDGYAFELWGQGTLVTVSS

SEQ ID NO: 68 - protein, 120 aa, Oryctolagus cuniculus
CQSLEESGGRLVTPGTPLTLTCTVSGIDLNNDYMTWVRQAPGKGLEWIGIFYVATEITWYASWAKGRFTISKTSTTVDLKITSPTTEDTATYFCGRDGGYTGDGYAFELWGQGTPVTVSS

SEQ ID NO: 69 - protein, 120 aa, Oryctolagus cuniculus
SQSLEESGGRLVTPGTPLTLTCTVSGIDLNNDYMTWVRQAPGKGLEWIGIFYVATEITWYASWAKGRFTISKTSTTVDLKITSPTTEDTATYFCGRDGGYTGDGYAFELWGQGTLVTVSS

SEQ ID NO: 70 - protein, 120 aa, Oryctolagus cuniculus
CQSLEESGGRLVTPGASLTLTCTVSGIDLNNDYMTWVRQAPGKGLEWIGIFYVATEITWYASWAKGRFTISKTSTTVDLKITSPTTEDTATYFCGRDGGYTGDGYAFELWGQGTLVTVSS

SEQ ID NO: 71 - protein, 120 aa, Oryctolagus cuniculus
CQSLEESGGRLVTPGTPLTLTCTVSGIDLNNDYMTWVRQAPGKGLEWIGIFYVATEITWYASWAKGRFTISKTSTTVDLKITSTTTEDTATYFCGRDGGYTGDGYAFELWGQGTLVTVSS

SEQ ID NO: 72 - protein, 120 aa, Oryctolagus cuniculus
CQSLEESGGDLVKPGASLTLTCTASGIDLNNDYMTWVRQAPGKGLEWIGIFYVATEITWYASWAKGRFTISKTSTTVDLKITRPTTEDTATYICGRDGGYTGDGYAFELWGQGTLVTVSS

SEQ ID NO: 73 - protein, 120 aa, Oryctolagus cuniculus
CQSLEESGGRLVTPGTPLTLTCTVSGIDLNNDYMTWVRQAPGKGLEWIGIFYVATEITWYASWAKGRFTIAKTSTTVDLKITSPTTEDTATYFCGRDGGYTGDGYAFELWGQGTLVTVSS

SEQ ID NO: 74 - protein, 120 aa, Oryctolagus cuniculus
CQSLEESGGRLVTPGTPLTLTCTVSGIDLTNDYMTWVRQAPGKGLEWIGIFYVATEITWYASWAKGRFTISKTSTTVDLKITSPTTEDTATYFCGRDGGYTGDGYAFELWGQGTLVTVSS

SEQ ID NO: 75 - protein, 120 aa, Oryctolagus cuniculus
CQSLEESGGRLVTPGTPLTLTCAVSGIDLNNDYMTWVRQAPGKGLEWIGIFYVATEITWYASWAKGRFTISKTSTTVDLKITSPTTEDTATYFCGRDGGYTGDGYAFELWGQGTLVTVSS

SEQ ID NO: 76 - protein, 120 aa, Oryctolagus cuniculus
CQSLEESGGRLVTPGTPLTLTCTVSGIDLNNDYMTWVRQAPGKGLEWIGIFYVETEITWYASWAKGRFTISKTSTTVDLKITSPTTEDTATYFCGRDGGYTGDGYAFELWGQGTLVTVSS

SEQ ID NO: 77 - protein, 120 aa, Oryctolagus cuniculus
CQSLEESGGRLVTPGTPLTLTCTVSGIDLNNDYMTWVRQAPGKGLEWIGIFYVATEITWYASWTKGRFTISKTSTTVDLKITSPTTEDTATYFCGRDGGYTGDGYAFELWGQGTLVTVSS

SEQ ID NO: 78 - protein, 120 aa, Oryctolagus cuniculus
CQSLEESGGRLVTPGTPLTLTCTVSGIDLNNDYMTWVRQAPGKGLEWIGIFYVATEITWYASWAKGRFTISKTSTAVDLKITSPTTEDTATYFCGRDGGYTGDGYAFELWGQGTLVTVSS

SEQ ID NO: 79 - protein, 120 aa, Oryctolagus cuniculus
CQSLEESGGRLVTPGTPLTLTCTVSGIDLNDDYMTWVRQAPGKGLEWIGIFYVATEITWYASWAKGRFTISKTSTTVDLKITSPTTEDTATYFCGRDGGYTGDGYAFELWGQGTLVTVSS

SEQ ID NO: 80 - protein, 120 aa, Oryctolagus cuniculus
CQSLEESGGRLVTPWTPLTLTCTVSGIDLNNDYMTWVRQAPGKGLEWIGIFYVATEITWYASWAKGRFTISKTSTTVDLKITSPTTEDTATYFCGRDGGYTGDGYAFELWGQGTLVTVSS